European Patent Application EP 4 726 048 A1, published April 15, 2026. Title: MICROORGANISMS FOR PRODUCING L-CITRULLINE AND PROCESS FOR PRODUCING L-CITRULLINE USING THE SAME. Applicant: 씨제이제일제당 (주). Application KR. The sequence listing filed with the application follows.

SEQUENCE LISTING (18 sequences)

SEQ ID NO: 1 - protein, 399 aa, Corynebacterium glutamicum
MGLWIDATAGVAGDMLLGALIDAGAELEKSNRLLKPLSLVTCFVLLRAEEVVRQGQRGIKLHVEAQHEHHHHRHLSTIKELLVNADIPAQTKQDALGVFELIAIAEGKVHGIEPEKIHFHEVGAWDSIADIVGVCEAIRQLNPGLIAASPIALGFGRIKAAHGDIPVPVPAVAELVKGWPTQTGALMESTEPVGELATPTGVALIRHFATQDGPFPGGIINEVGIGAGTKDTAGRPNVVRAVLFSTSGKAASNPDTRTLVQLEANVDDQDPRLWPGVIESLFAAGAVAAWLTPILMKKGRPAHTVSALVDSSEVEAVKTALFAATTTFGVRSWEVQREGLDRRFEQVEVDGRTINIKIGSRNGHDISAQPEFEDIRSAAVALGISEREVVARIPQGTTE

SEQ ID NO: 2 - DNA, 1193 bp, Corynebacterium glutamicum
  source 1..1193: mol_type = genomic DNA
atggggctgtggatcgatgcaaccgctggcgttgcaggggatatgttgctgggagcactcattgatgcaggtgcagaactagaaaaatccaacaggttgttgaagccgttatccctggtgacgtgcttttgagagcagaagaggtagtgcgccaaggccaacgaggcatcaaactacatgtagaagcacaacatgaacaccaccatcaccgccatttgagcaccattaaagaactgcttgtcaatgctgacatccctgcacaaaccaagcaggatgccttaggcgtttttgaactcatcgctatcgctgaaggaaaagtccacggcatcgagccggagaaaatccacttccatgaggtaggagcttgggattccatcgcagacattgtgggtgtgtgcgaagcgatcaggcagcttaacccaggtttgattgctgcatctccgattgctttaggattcggacgcatcaaggcagctcacggagacattccagtgccagttccagcagtggcagagctggtgaaaggctggcccacccaaaccggagctcttatggagagcaccgaacctgttggtgaattagccaccccaactggtgttgcgttgatccgtcactttgccacccaagatggccctttcccaggtggcatcatcaatgaagtcggtatcggcgcaggaactaaggacaccgcagggcgtcccaatgtggtgcgcgcggtcctgttcagcacctccggtaaggctgcctcaaacccagacacccgtaccctcgtgcaattggaagccaacgttgatgatcaagacccacggctgtggccaggagtaatagagagcctctttgccgctggcgcagtagctgcatggctgactccaattttgatgaagaagggccgtcctgcacatacggtgtcagcattggtggatagctccgaggtggaagcagtgaaaaccgcattatttgcagccaccacgacttttggggtcagatcatgggaagtccagcgagaagggttggatcgtcgtttcgaacaagtcgaggtggacggacgcaccatcaacatcaagattggctcccgaaatggccacgacatcagtgcacagcccgagtttgaagatattcggtctgcagcggtggccttgggaatttcagagagggaagttgtggcaagaattccgcaaggcaccactgagtaa

SEQ ID NO: 3 - DNA, 34 bp, synthetic construct
  source 1..34: mol_type = other DNA
tcggtacccggggatccccccagtaacaagtgct

SEQ ID NO: 4 - DNA, 34 bp, synthetic construct
  source 1..34: mol_type = other DNA
cttttggttgtattctcgcttcttcaaatcagtt

SEQ ID NO: 5 - DNA, 34 bp, synthetic construct
  source 1..34: mol_type = other DNA
gagaatacaaccaaaaggtcgactgcttctaatt

SEQ ID NO: 6 - DNA, 34 bp, synthetic construct
  source 1..34: mol_type = other DNA
tgcaggtcgactctagaaggccatcatcgacacc

SEQ ID NO: 7 - DNA, 20 bp, synthetic construct
  source 1..20: mol_type = other DNA
tattacgccagctggcgaaa

SEQ ID NO: 8 - DNA, 20 bp, synthetic construct
  source 1..20: mol_type = other DNA
gctttacactttatgcttcc

SEQ ID NO: 9 - DNA, 36 bp, synthetic construct
  source 1..36: mol_type = other DNA
cggtacccggggatccctcgtgcggaattcgtggag

SEQ ID NO: 10 - DNA, 20 bp, synthetic construct
  source 1..20: mol_type = other DNA
atccagcagcaattcagaca

SEQ ID NO: 11 - DNA, 37 bp, synthetic construct
  source 1..37: mol_type = other DNA
ctgaattgctgctggattaaggcatcgatatcaccca

SEQ ID NO: 12 - DNA, 36 bp, synthetic construct
  source 1..36: mol_type = other DNA
atgcctgcaggtcgacccttcattttaagttccttg

SEQ ID NO: 13 - DNA, 33 bp, synthetic construct
  source 1..33: mol_type = other DNA
cggtacccggggatccttcatcgatagggtggg

SEQ ID NO: 14 - DNA, 34 bp, synthetic construct
  source 1..34: mol_type = other DNA
gtactcctcagcttactcatcctttgcatcaaca

SEQ ID NO: 15 - DNA, 34 bp, synthetic construct
  source 1..34: mol_type = other DNA
agtaagctgaggagtactgcctgccaaccatcaa

SEQ ID NO: 16 - DNA, 34 bp, synthetic construct
  source 1..34: mol_type = other DNA
atgcctgcaggtcgaccgactggcttgccaccct

SEQ ID NO: 17 - protein, 43 aa, Corynebacterium glutamicum
MGLWIDATAGVAGDMLLGALIDAGAELEKSNRLLKPLSLVTCF

SEQ ID NO: 18 - protein, 356 aa, Corynebacterium glutamicum
VLLRAEEVVRQGQRGIKLHVEAQHEHHHHRHLSTIKELLVNADIPAQTKQDALGVFELIAIAEGKVHGIEPEKIHFHEVGAWDSIADIVGVCEAIRQLNPGLIAASPIALGFGRIKAAHGDIPVPVPAVAELVKGWPTQTGALMESTEPVGELATPTGVALIRHFATQDGPFPGGIINEVGIGAGTKDTAGRPNVVRAVLFSTSGKAASNPDTRTLVQLEANVDDQDPRLWPGVIESLFAAGAVAAWLTPILMKKGRPAHTVSALVDSSEVEAVKTALFAATTTFGVRSWEVQREGLDRRFEQVEVDGRTINIKIGSRNGHDISAQPEFEDIRSAAVALGISEREVVARIPQGTTE